European Patent Application EP 4 248 998 A1, published September 27, 2023. Title: 用于控制生物体内热量产生的组合物、方法及用途. Applicant: 广东暨安特博生物科技有限公司. The sequence listing filed with the application follows.

SEQUENCE LISTING (30 sequences)

SEQ ID NO: 1 - DNA, 19 bp, synthetic construct
  source 1..19: mol_type = other DNA; note = primer; note (original language) = 引物; organism (original language) = 合成构建体
tcattatgccgaggatttg

SEQ ID NO: 2 - DNA, 18 bp, synthetic construct
  source 1..18: mol_type = other DNA; note = primer; note (original language) = 引物; organism (original language) = 合成构建体
gcctcccatctccttcat

SEQ ID NO: 3 - DNA, 20 bp, synthetic construct
  source 1..20: mol_type = other DNA; note = primer; note (original language) = 引物; organism (original language) = 合成构建体
ctactgaacttcggggtgat

SEQ ID NO: 4 - DNA, 19 bp, synthetic construct
  source 1..19: mol_type = other DNA; note = primer; note (original language) = 引物; organism (original language) = 合成构建体
caggcttgtcactcgaatt

SEQ ID NO: 5 - DNA, 20 bp, synthetic construct
  source 1..20: mol_type = other DNA; note = primer; note (original language) = 引物; organism (original language) = 合成构建体
tccagttgccttcttgggac

SEQ ID NO: 6 - DNA, 21 bp, synthetic construct
  source 1..21: mol_type = other DNA; note = primer; note (original language) = 引物; organism (original language) = 合成构建体
gtgtaattaagcgccgacttg

SEQ ID NO: 7 - DNA, 27 bp, synthetic construct
  source 1..27: mol_type = other DNA; note = primer; note (original language) = 引物; organism (original language) = 合成构建体
ggctggtgcaaagaaacatggacttga

SEQ ID NO: 8 - DNA, 25 bp, synthetic construct
  source 1..25: mol_type = other DNA; note = primer; note (original language) = 引物; organism (original language) = 合成构建体
tgcagacagagacgccattccacat

SEQ ID NO: 9 - DNA, 25 bp, synthetic construct
  source 1..25: mol_type = other DNA; note = primer; note (original language) = 引物; organism (original language) = 合成构建体
caaccaacaagtgatattctccatg

SEQ ID NO: 10 - DNA, 21 bp, synthetic construct
  source 1..21: mol_type = other DNA; note = primer; note (original language) = 引物; organism (original language) = 合成构建体
gatccacactctccagctgca

SEQ ID NO: 11 - DNA, 21 bp, synthetic construct
  source 1..21: mol_type = other DNA; note = primer; note (original language) = 引物; organism (original language) = 合成构建体
gaaaactccatgcttgaagaa

SEQ ID NO: 12 - DNA, 21 bp, synthetic construct
  source 1..21: mol_type = other DNA; note = primer; note (original language) = 引物; organism (original language) = 合成构建体
tctttcagtgatgtggacttg

SEQ ID NO: 13 - DNA, 20 bp, synthetic construct
  source 1..20: mol_type = other DNA; note = primer; note (original language) = 引物; organism (original language) = 合成构建体
tcaccgagctctgttgacaa

SEQ ID NO: 14 - DNA, 20 bp, synthetic construct
  source 1..20: mol_type = other DNA; note = primer; note (original language) = 引物; organism (original language) = 合成构建体
ccacacttctctttttggcg

SEQ ID NO: 15 - DNA, 21 bp, synthetic construct
  source 1..21: mol_type = other DNA; note = primer; note (original language) = 引物; organism (original language) = 合成构建体
tgagcaacatcacacaagacc

SEQ ID NO: 16 - DNA, 19 bp, synthetic construct
  source 1..19: mol_type = other DNA; note = primer; note (original language) = 引物; organism (original language) = 合成构建体
ggccttgcggttacagagg

SEQ ID NO: 17 - DNA, 21 bp, synthetic construct
  source 1..21: mol_type = other DNA; note = primer; note (original language) = 引物; organism (original language) = 合成构建体
actgccacacctccagtcatt

SEQ ID NO: 18 - DNA, 21 bp, synthetic construct
  source 1..21: mol_type = other DNA; note = primer; note (original language) = 引物; organism (original language) = 合成构建体
ctttgcctcactcaggattgg

SEQ ID NO: 19 - DNA, 20 bp, synthetic construct
  source 1..20: mol_type = other DNA; note = primer; note (original language) = 引物; organism (original language) = 合成构建体
gaaccatgaagccaacgact

SEQ ID NO: 20 - DNA, 20 bp, synthetic construct
  source 1..20: mol_type = other DNA; note = primer; note (original language) = 引物; organism (original language) = 合成构建体
gcgaagttcacagtggttcc

SEQ ID NO: 21 - DNA, 21 bp, synthetic construct
  source 1..21: mol_type = other DNA; note = primer; note (original language) = 引物; organism (original language) = 合成构建体
tgctcttctgtatcgcccagt

SEQ ID NO: 22 - DNA, 21 bp, synthetic construct
  source 1..21: mol_type = other DNA; note = primer; note (original language) = 引物; organism (original language) = 合成构建体
gccgtgttaaggaatctgctg

SEQ ID NO: 23 - DNA, 19 bp, synthetic construct
  source 1..19: mol_type = other DNA; note = primer; note (original language) = 引物; organism (original language) = 合成构建体
cagcacggtgaagccattc

SEQ ID NO: 24 - DNA, 17 bp, synthetic construct
  source 1..17: mol_type = other DNA; note = primer; note (original language) = 引物; organism (original language) = 合成构建体
gcgtgcatccgcttgtg

SEQ ID NO: 25 - DNA, 20 bp, synthetic construct
  source 1..20: mol_type = other DNA; note = primer; note (original language) = 引物; organism (original language) = 合成构建体
gaatcattatgacggcagca

SEQ ID NO: 26 - DNA, 22 bp, synthetic construct
  source 1..22: mol_type = other DNA; note = primer; note (original language) = 引物; organism (original language) = 合成构建体
tcatgtacaccgtgatgtggta

SEQ ID NO: 27 - DNA, 21 bp, synthetic construct
  source 1..21: mol_type = other DNA; note = primer; note (original language) = 引物; organism (original language) = 合成构建体
tccgcgttctcatgtaggtct

SEQ ID NO: 28 - DNA, 21 bp, synthetic construct
  source 1..21: mol_type = other DNA; note = primer; note (original language) = 引物; organism (original language) = 合成构建体
ggacctgatgcaaccctatga

SEQ ID NO: 29 - DNA, 24 bp, synthetic construct
  source 1..24: mol_type = other DNA; note = primer; note (original language) = 引物; organism (original language) = 合成构建体
ctggttctggtatggtttggggtt

SEQ ID NO: 30 - DNA, 24 bp, synthetic construct
  source 1..24: mol_type = other DNA; note = primer; note (original language) = 引物; organism (original language) = 合成构建体
tgaaagaactcaacagtgggccgg